European Patent Specification EP 3 630 793 B1, published July 10, 2024. Title: A RECOMBINANT PROTEIN. Applicant: GE Healthcare BioProcess R&D AB. The sequence listing filed with the application follows.

SEQUENCE LISTING (129 sequences)

SEQ ID NO: 1 - protein, 51 aa, Staphylococcus aureus
AQQNAFYQVLNMPNLNADQRNGFIQSLKDDPSQSANVLGEAQKLNDSQAPK

SEQ ID NO: 2 - protein, 61 aa, Staphylococcus aureus
ADAQQNKFNKDQQSAFYEILNMPNLNEEQRNGFIQSLKDDPSQSTNVLGEAKKLNESQAPK

SEQ ID NO: 3 - protein, 58 aa, Staphylococcus aureus
ADNNFNKEQQNAFYEILNMPNLNEEQRNGFIQSLKDDPSQSANLLAEAKKLNESQAPK

SEQ ID NO: 4 - protein, 58 aa, Staphylococcus aureus [sequence omitted]

SEQ ID NO: 5 - protein, 58 aa, Staphylococcus aureus
ADNKFNKEQQNAFYEILHLPNLTEEQRNGFIQSLKDDPSVSKEILAEAKKLNDAQAPK

SEQ ID NO: 6 - protein, 58 aa, Artificial Sequence [sequence omitted]

SEQ ID NO: 7 - protein, 58 aa, Artificial Sequence [sequence omitted]

SEQ ID NO: 8 - protein, 58 aa, Artificial Sequence
  Protein A domain variant
VDAKFDKEAQEAFYEILHLPNLTEEQRNAFIQSLKDDPSVSKAILAEAKKLNDAQAPK

SEQ ID NO: 9 - protein, 47 aa, Staphylococcus aureus
QQNAFYEILHLPNLTEEQRNGFIQSLKDDPSVSKEILAEAKKLNDAQ

SEQ ID NO: 10 - protein, 47 aa, Artificial Sequence; identical to SEQ ID NO: 9
  Protein A domain variant

SEQ ID NO: 11 - protein, 47 aa, Artificial Sequence
  Protein A domain variant
AQEAFYEILHLPNLTEEQRNAFIQSLKDDPSVSKAILAEAKKLNDAQ

SEQ ID NO: 12 - protein, 233 aa, Artificial Sequence
  Multimer of protein A domain variants
VDAKFDKEQQNAFYEILHLPNLTEEQRNAFIQSLKDDPSQSANLLAEAKKLNDAQAPKVDAKFDKEQQNAFYEILHLPNLTEEQRNAFIQSLKDDPSQSANLLAEAKKLNDAQAPKVDAKFDKEQQNAFYEILHLPNLTEEQRNAFIQSLKDDPSQSANLLAEAKKLNDAQAPKVDAKFDKEQQNAFYEILHLPNLTEEQRNAFIQSLKDDPSQSANLLAEAKKLNDAQAPKC

SEQ ID NO: 13 - protein, 349 aa, Artificial Sequence
  Multimer of protein A domain variants
VDAKFDKEAQEAFYEILHLPNLTEEQRNAFIQSLKDDPSVSKAILAEAKKLNDAQAPKVDAKFDKEAQEAFYEILHLPNLTEEQRNAFIQSLKDDPSVSKAILAEAKKLNDAQAPKVDAKFDKEAQEAFYEILHLPNLTEEQRNAFIQSLKDDPSVSKAILAEAKKLNDAQAPKVDAKFDKEAQEAFYEILHLPNLTEEQRNAFIQSLKDDPSVSKAILAEAKKLNDAQAPKVDAKFDKEAQEAFYEILHLPNLTEEQRNAFIQSLKDDPSVSKAILAEAKKLNDAQAPKVDAKFDKEAQEAFYEILHLPNLTEEQRNAFIQSLKDDPSVSKAILAEAKKLNDAQAPKC

SEQ ID NO: 14 - protein, 21 aa, Escherichia coli
MKKTAIAIAVALAGFATVAQA

SEQ ID NO: 15 - protein, 19 aa, Escherichia coli
MKKIWLALAGLVLAFSASA

SEQ ID NO: 16 - protein, 12 aa, Escherichia coli
AQKDQTWYTGGT

SEQ ID NO: 17 - protein, 12 aa, Escherichia coli
AQYEDGKQYTGT

SEQ ID NO: 18 - protein, 12 aa, Staphylococcus aureus
AQHDEAQQEAGT

SEQ ID NO: 19 - protein, 12 aa, Escherichia coli
AQGGGSGGGSGT

SEQ ID NO: 20 - DNA, 33 bp, Escherichia coli
gcagaaagatcagacctggtacaccggcggtac

SEQ ID NO: 21 - DNA, 29 bp, Escherichia coli
cgccggtgtaccaggtctgatctttctgc

SEQ ID NO: 22 - DNA, 33 bp, Escherichia coli
gcagcatgatgaagcgcagcaggaagcgggtac

SEQ ID NO: 23 - DNA, 29 bp, Escherichia coli
ccgcttcctgctgcgcttcatcatgctgc

SEQ ID NO: 24 - DNA, 33 bp, Escherichia coli
gcagtatgaagatggcaaacagtacaccggtac

SEQ ID NO: 25 - DNA, 29 bp, Escherichia coli
cggtgtactgtttgccatcttcatactgc

SEQ ID NO: 26 - DNA, 33 bp, Escherichia coli
gcagggtggcggttctggcggtggcagcggtac

SEQ ID NO: 27 - DNA, 29 bp, Escherichia coli
cgctgccaccgccagaaccgccaccctgc

SEQ ID NO: 28 - protein, 4 aa, Staphylococcus aureus
AQGT

SEQ ID NO: 29 - protein, 11 aa, Artificial Sequence
  Spacer variant
AQYEDGKQYGT

SEQ ID NO: 30 - protein, 10 aa, Artificial Sequence
  Spacer variant
AQYEDGKQGT

SEQ ID NO: 31 - protein, 9 aa, Artificial Sequence
  Spacer variant
AQYEDGKGT

SEQ ID NO: 32 - protein, 8 aa, Artificial Sequence
  Spacer variant
AQYEDGGT

SEQ ID NO: 33 - protein, 16 aa, Artificial Sequence
  Spacer variant
AQYEDGKQYTTLEKGT

SEQ ID NO: 34 - protein, 20 aa, Artificial Sequence
  Spacer variant
AQYEDGKQYTTLEKPVAGGT

SEQ ID NO: 35 - protein, 10 aa, Artificial Sequence
  Spacer variant
AQYEDGKQYT

SEQ ID NO: 36 - protein, 8 aa, Artificial Sequence
  Spacer variant
AQYEDGKQ

SEQ ID NO: 37 - protein, 12 aa, Artificial Sequence
  Spacer variant
AQYEDGKQYTET

SEQ ID NO: 38 - protein, 12 aa, Artificial Sequence
  Spacer variant
AQYEDGKQYTDT

SEQ ID NO: 39 - protein, 12 aa, Artificial Sequence
  Spacer variant
AQYEDGKQYTAT

SEQ ID NO: 40 - protein, 12 aa, Artificial Sequence
  Spacer variant
AQYEDGKQYEDT

SEQ ID NO: 41 - protein, 12 aa, Artificial Sequence
  Spacer variant
AQRRRRRRRRGT

SEQ ID NO: 42 - protein, 12 aa, Artificial Sequence
  Spacer variant
AQKKKKKKKKGT

SEQ ID NO: 43 - protein, 12 aa, Artificial Sequence
  Spacer variant
AQHHHHHHHHGT

SEQ ID NO: 44 - protein, 10 aa, Artificial Sequence
  Spacer variant
AQHHHHHHGT

SEQ ID NO: 45 - protein, 8 aa, Artificial Sequence
  Spacer variant
AQHHHHGT

SEQ ID NO: 46 - protein, 12 aa, Artificial Sequence
  Spacer variant
AQWSHPQFEKGT

SEQ ID NO: 47 - protein, 12 aa, Staphylococcus aureus
AQHDEAQQEAGT

SEQ ID NO: 48 - protein, 58 aa, Artificial Sequence
  Protein A domain variant
VDAKFDKEAQEAFYEILHLPNLTEEQRNGFIQSLKDDPSVSKAILAEAKKLNDAQAPK

SEQ ID NO: 49 - protein, 58 aa, Artificial Sequence
  Protein A domain variant
VDAKFDKEAQEAFYEILHLPNLTEEQRNSFIQSLKDDPSVSKAILAEAKKLNDAQAPK

SEQ ID NO: 50 - protein, 58 aa, Artificial Sequence
  Protein A domain variant
VDAKFDKEAQEAFYEILHLPNLTEEQRNYFIQSLKDDPSVSKAILAEAKKLNDAQAPK

SEQ ID NO: 51 - protein, 58 aa, Artificial Sequence
  Protein A domain variant
VDAKFDKEAQEAFYEILHLPNLTEEQRNQFIQSLKDDPSVSKAILAEAKKLNDAQAPK

SEQ ID NO: 52 - protein, 58 aa, Artificial Sequence
  Protein A domain variant
VDAKFDKEAQEAFYEILHLPNLTEEQRNTFIQSLKDDPSVSKAILAEAKKLNDAQAPK

SEQ ID NO: 53 - protein, 58 aa, Artificial Sequence
  Protein A domain variant
VDAKFDKEAQEAFYEILHLPNLTEEQRNNFIQSLKDDPSVSKAILAEAKKLNDAQAPK

SEQ ID NO: 54 - protein, 58 aa, Artificial Sequence
  Protein A domain variant
VDAKFDKEAQEAFYEILHLPNLTEEQRNFFIQSLKDDPSVSKAILAEAKKLNDAQAPK

SEQ ID NO: 55 - protein, 58 aa, Artificial Sequence
  Protein A domain variant
VDAKFDKEAQEAFYEILHLPNLTEEQRNLFIQSLKDDPSVSKAILAEAKKLNDAQAPK

SEQ ID NO: 56 - protein, 58 aa, Artificial Sequence
  Protein A domain variant
VDAKFDKEAQEAFYEILHLPNLTEEQRNWFIQSLKDDPSVSKAILAEAKKLNDAQAPK

SEQ ID NO: 57 - protein, 58 aa, Artificial Sequence
  Protein A domain variant
VDAKFDKEAQEAFYEILHLPNLTEEQRNIFIQSLKDDPSVSKAILAEAKKLNDAQAPK

SEQ ID NO: 58 - protein, 58 aa, Artificial Sequence
  Protein A domain variant
VDAKFDKEAQEAFYEILHLPNLTEEQRNMFIQSLKDDPSVSKAILAEAKKLNDAQAPK

SEQ ID NO: 59 - protein, 58 aa, Artificial Sequence
  Protein A domain variant
VDAKFDKEAQEAFYEILHLPNLTEEQRNVFIQSLKDDPSVSKAILAEAKKLNDAQAPK

SEQ ID NO: 60 - protein, 58 aa, Artificial Sequence
  Protein A domain variant
VDAKFDKEAQEAFYEILHLPNLTEEQRNDFIQSLKDDPSVSKAILAEAKKLNDAQAPK

SEQ ID NO: 61 - protein, 58 aa, Artificial Sequence
  Protein A domain variant
VDAKFDKEAQEAFYEILHLPNLTEEQRNEFIQSLKDDPSVSKAILAEAKKLNDAQAPK

SEQ ID NO: 62 - protein, 58 aa, Artificial Sequence
  Protein A domain variant
VDAKFDKEAQEAFYEILHLPNLTEEQRNHFIQSLKDDPSVSKAILAEAKKLNDAQAPK

SEQ ID NO: 63 - protein, 58 aa, Artificial Sequence
  Protein A domain variant
VDAKFDKEAQEAFYEILHLPNLTEEQRNRFIQSLKDDPSVSKAILAEAKKLNDAQAPK

SEQ ID NO: 64 - protein, 58 aa, Artificial Sequence
  Protein A domain variant
VDAKFDKEAQEAFYEILHLPNLTEEQRNKFIQSLKDDPSVSKAILAEAKKLNDAQAPK

SEQ ID NO: 65 - protein, 113 aa, Artificial Sequence
  Dimer of protein A domain variants
VDAKFDKEAQEAFYEILHLPNLTEEQRNAFIQSLKDDPSVSKAILAEAKKLNDAQAPKVFDKEAQEAFYEILHLPNLTEEQRNAFIQSLKDDPSVSKAILAEAKKLNDAQAPK

SEQ ID NO: 66 - protein, 113 aa, Artificial Sequence
  Dimer of protein A domain variants
VDAKFDKEAQEAFYEILHLPNLTEEQRNAFIQSLKDDPSVSKAILAEAKKLNDAQAPAKFDKEAQEAFYEILHLPNLTEEQRNAFIQSLKDDPSVSKAILAEAKKLNDAQAPK

SEQ ID NO: 67 - protein, 111 aa, Artificial Sequence
  Dimer of protein A domain variants
VDAKFDKEAQEAFYEILHLPNLTEEQRNAFIQSLKDDPSVSKAILAEAKKLNDAQAKFDKEAQEAFYEILHLPNLTEEQRNAFIQSLKDDPSVSKAILAEAKKLNDAQAPK

SEQ ID NO: 68 - protein, 111 aa, Artificial Sequence
  Dimer of protein A domain variants
VDAKFDKEAQEAFYEILHLPNLTEEQRNAFIQSLKDDPSVSKAILAEAKKLNDAQAPKVDAAQEAFYEILHLPNLTEEQRNAFIQSLKDDPSVSKAILAEAKKLNDAQAPK

SEQ ID NO: 69 - protein, 113 aa, Artificial Sequence
  Dimer of protein A domain variants
VDAKFDKEAQEAFYEILHLPNLTEEQRNAFIQSLKDDPSVSKAILAEAKKLNDAQVDAKFDKEAQEAFYEILHLPNLTEEQRNAFIQSLKDDPSVSKAILAEAKKLNDAQAPK

SEQ ID NO: 70 - protein, 113 aa, Artificial Sequence
  Dimer of protein A domain variants
VDAKFDKEAQEAFYEILHLPNLTEEQRNAFIQSLKDDPSVSKAILAEAKKLNDAQAPKKFDKEAQEAFYEILHLPNLTEEQRNAFIQSLKDDPSVSKAILAEAKKLNDAQAPK

SEQ ID NO: 71 - protein, 108 aa, Artificial Sequence
  Dim er of protein A domain variants
VDAKFDKEAQEAFYEILHLPNLTEEQRNAFIQSLKDDPSVSKAILAEAKKLNDAQAPKAQEAFYEILHLPNLTEEQRNAFIQSLKDDPSVSKAILAEAKKLNDAQAPK

SEQ ID NO: 72 - protein, 124 aa, Artificial Sequence
  Dimer of protein A domain variants
VDAKFDKEAQEAFYEILHLPNLTEEQRNAFIQSLKDDPSVSKAILAEAKKLNDAQAPKYEDGKQYTVDAKFDKEAQEAFYEILHLPNLTEEQRNAFIQSLKDDPSVSKAILAEAKKLNDAQAPK

SEQ ID NO: 73 - protein, 120 aa, Artificial Sequence
  Dimer of protein A domain variants
VDAKFDKEAQEAFYEILHLPNLTEEQRNAFIQSLKDDPSVSKAILAEAKKLNDAQAPKYEDGVDAKFDKEAQEAFYEILHLPNLTEEQRNAFIQSLKDDPSVSKAILAEAKKLNDAQAPK

SEQ ID NO: 74 - protein, 57 aa, Artificial Sequence
  Protein A domain variant
VDAKFDKEQEAFYEILHLPNLTEEQRNAFIQSLKDDPSVSKAILAEAKKLNDAQAPK

SEQ ID NO: 75 - protein, 57 aa, Artificial Sequence
  Protein A domain variant
VDAKFDKEAQEAFYEILHLPNLTEEQRNAFIQSLKDDPSSKAILAEAKKLNDAQAPK

SEQ ID NO: 76 - protein, 57 aa, Artificial Sequence
  Protein A domain variant
VDAKFDKEAQEAFYEILHLPNLTEEQRNAFIQSLKDDPSVSAILAEAKKLNDAQAPK

SEQ ID NO: 77 - protein, 57 aa, Artificial Sequence
  Protein A domain variant
VDAKFDKEAQEAFYEILHLPNLTEEQRNAFIQSLKDDPSVSKILAEAKKLNDAQAPK

SEQ ID NO: 78 - protein, 57 aa, Artificial Sequence
  Protein A domain variant
VDAKFDKEAQEAFYEILHLPNLTEEQRNAFIQSLKDDPSVSKALAEAKKLNDAQAPK

SEQ ID NO: 79 - protein, 58 aa, Artificial Sequence
  Protein A domain variant
VDAKFDKEAQNFFYEILHLPNLTEEQRNAFIQSLKDDPSVSKAILAEAKKLNDAQAPK

SEQ ID NO: 80 - protein, 58 aa, Artificial Sequence
  Protein A domain variant
VDAKFDKEAQNYFYEILHLPNLTEEQRNAFIQSLKDDPSVSKAILAEAKKLNDAQAPK

SEQ ID NO: 81 - protein, 58 aa, Artificial Sequence
  Protein A domain variant
VDAKFDKEAQNKFYEILHLPNLTEEQRNAFIQSLKDDPSVSKAILAEAKKLNDAQAPK

SEQ ID NO: 82 - protein, 58 aa, Artificial Sequence
  Protein A domain variant
VDAKFDKEAQNRFYEILHLPNLTEEQRNAFIQSLKDDPSVSKAILAEAKKLNDAQAPK

SEQ ID NO: 83 - protein, 58 aa, Artificial Sequence
  Protein A domain variant
VDAKFDKEAQEAFYEILHLPNFTEEQRNAFIQSLKDDPSVSKAILAEAKKLNDAQAPK

SEQ ID NO: 84 - protein, 58 aa, Artificial Sequence
  Protein A domain variant
VDAKFDKEAQEAFYEILHLPNLTEEQRNAFIQSLKDDPSVSKNFLAEAKKLNDAQAPK

SEQ ID NO: 85 - protein, 58 aa, Artificial Sequence
  Protein A domain variant
VDAKFDKEAQEAFYEILHLPNLTEEQRNAFIQSLKDDPSVSKNYLAEAKKLNDAQAPK

SEQ ID NO: 86 - protein, 58 aa, Artificial Sequence
  Protein A domain variant
VDAKFDKEAQEAFYEILHLPNLTEEQRNAFIQSLKDDPSVSKNWLAEAKKLNDAQAPK

SEQ ID NO: 87 - protein, 58 aa, Artificial Sequence
  Protein A domain variant
VDAKFDKEAQEAFYEILHLPNLTEEQRNAFIQSLKDDPSVSKNRLAEAKKLNDAQAPK

SEQ ID NO: 88 - protein, 58 aa, Artificial Sequence
  Protein A domain variant
VDAKFDKEAQEAFYEILHLPNLTEEQRNAFIQSLKDDPSVSKNKLAEAKKLNDAQAPK

SEQ ID NO: 89 - protein, 58 aa, Artificial Sequence
  Protein A domain variant
VDAKFDKEAQEAFYEILHLPNLTEEQRNAFIQSLKDDPSVSKAILAEAKKLNFAQAPK

SEQ ID NO: 90 - protein, 58 aa, Artificial Sequence
  Protein A domain variant
VDAKFDKEAQEAFYEILHLPNLTEEQRNAFIQSLKDDPSVSKAILAEAKKLNYAQAPK

SEQ ID NO: 91 - protein, 58 aa, Artificial Sequence
  Protein A domain variant
VDAKFDKEAQEAFYEILHLPNLTEEQRNAFIQSLKDDPSVSKAILAEAKKLNWAQAPK

SEQ ID NO: 92 - protein, 58 aa, Artificial Sequence
  Protein A domain variant
VDAKFDKEAQEAFYEILHLPNLTEEQRNAFIQSLKDDPSVSKAILAEAKKLNKAQAPK

SEQ ID NO: 93 - protein, 58 aa, Artificial Sequence
  Protein A domain variant
VDAKFDKEAQEAFYEILHLPNLTEEQRNAFIQSLKDDPSVSKAILAEAKKLNRAQAPK

SEQ ID NO: 94 - DNA, 30 bp, Artificial Sequence
  Spacer variant
gcagtatgaagatggcaaacagtacggtac

SEQ ID NO: 95 - DNA, 26 bp, Artificial Sequence
  Spacer variant
cgtactgtttgccatcttcatactgc

SEQ ID NO: 96 - DNA, 27 bp, Artificial Sequence
  Spacer variant
gcagtatgaagatggcaaacagggtac

SEQ ID NO: 97 - DNA, 23 bp, Artificial Sequence
  Spacer variant
cctgtttgccatcttcatactgc

SEQ ID NO: 98 - DNA, 24 bp, Artificial Sequence
  Spacer variant
gcagtatgaagatggcaaaggtac

SEQ ID NO: 99 - DNA, 20 bp, Artificial Sequence
  Spacer variant
ctttgccatcttcatactgc

SEQ ID NO: 100 - DNA, 21 bp, Artificial Sequence
  Spacer variant
gcagtatgaagatggcggtac

SEQ ID NO: 101 - DNA, 17 bp, Artificial Sequence
  Spacer variant
cgccatcttcatactgc

SEQ ID NO: 102 - DNA, 30 bp, Artificial Sequence
  Spacer variant
gcagtatgaagatggcaaacagtacaccgt

SEQ ID NO: 103 - DNA, 32 bp, Artificial Sequence
  Spacer variant
ctacggtgtactgtttgccatcttcatactgc

SEQ ID NO: 104 - DNA, 24 bp, Artificial Sequence
  Spacer variant
gcagtatgaagatggcaaacaggt

SEQ ID NO: 105 - DNA, 26 bp, Artificial Sequence
  Spacer variant
ctacctgtttgccatcttcatactgc

SEQ ID NO: 106 - DNA, 36 bp, Artificial Sequence
  Spacer variant
gcagtatgaagatggcaaacagtacaccgaaaccgt

SEQ ID NO: 107 - DNA, 38 bp, Artificial Sequence
  Spacer variant
ctacggtttcggtgtactgtttgccatcttcatactgc

SEQ ID NO: 108 - DNA, 36 bp, Artificial Sequence
  Spacer variant
gcagtatgaagatggcaaacagtacaccgataccgt

SEQ ID NO: 109 - DNA, 38 bp, Artificial Sequence
  Spacer variant
ctacggtatcggtgtactgtttgccatcttcatactgc

SEQ ID NO: 110 - DNA, 36 bp, Artificial Sequence
  Spacer variant
gcagtatgaagatggcaaacagtacaccgcgaccgt

SEQ ID NO: 111 - DNA, 38 bp, Artificial Sequence
  Spacer variant
ctacggtcgcggtgtactgtttgccatcttcatactgc

SEQ ID NO: 112 - DNA, 36 bp, Artificial Sequence
  Spacer variant
gcagtatgaagatggcaaacagtacgaagataccgt

SEQ ID NO: 113 - DNA, 38 bp, Artificial Sequence
  Spacer variant
ctacggtatcttcgtactgtttgccatcttcatactgc

SEQ ID NO: 114 - DNA, 45 bp, Artificial Sequence
  Spacer variant
gcagtatgaagatggcaaacagtacaccaccctggaaaaaggtac

SEQ ID NO: 115 - DNA, 41 bp, Artificial Sequence
  Spacer variant
ctttttccagggtggtgtactgtttgccatcttcatactgc

SEQ ID NO: 116 - DNA, 57 bp, Artificial Sequence
  Spacer variant
gcagtatgaagatggcaaacagtacaccaccctggaaaaaccggtggcgggcggtac

SEQ ID NO: 117 - DNA, 53 bp, Artificial Sequence
  Spacer variant
cgcccgccaccggtttttccagggtggtgtactgtttgccatcttcatactgc

SEQ ID NO: 118 - DNA, 33 bp, Artificial Sequence
  Spacer variant
gcagcgccgtcgtcgccgtcgccgtcgtggtac

SEQ ID NO: 119 - DNA, 29 bp, Artificial Sequence
  Spacer variant
cacgacggcgacggcgacgacggcgctgc

SEQ ID NO: 120 - DNA, 33 bp, Artificial Sequence
  Spacer variant
gcagaagaagaaaaagaagaagaaaaagggtac

SEQ ID NO: 121 - DNA, 29 bp, Artificial Sequence
  Spacer variant
cctttttcttcttctttttcttcttctgc

SEQ ID NO: 122 - DNA, 33 bp, Artificial Sequence
  Spacer variant
gcagcatcaccaccatcaccatcaccatggtac

SEQ ID NO: 123 - DNA, 29 bp, Artificial Sequence
  Spacer variant
catggtgatggtgatggtggtgatgctgc

SEQ ID NO: 124 - DNA, 27 bp, Artificial Sequence
  Spacer variant
gcagcatcaccaccatcaccatggtac

SEQ ID NO: 125 - DNA, 23 bp, Artificial Sequence
  Spacer variant
catggtgatggtggtgatgctgc

SEQ ID NO: 126 - DNA, 21 bp, Artificial Sequence
  Spacer variant
gcagcatcaccaccatggtac

SEQ ID NO: 127 - DNA, 17 bp, Artificial Sequence
  Spacer variant
catggtggtgatgctgc

SEQ ID NO: 128 - DNA, 33 bp, Artificial Sequence
  Spacer variant
gcagtggagccatccgcagtttgaaaaaggtac

SEQ ID NO: 129 - DNA, 29 bp, Artificial Sequence
  Spacer variant
ctttttcaaactgcggatggctccactgc